European Patent Application EP 4 279 074 A1, published November 22, 2023. Title: Azolo compounds for treatment of fibrotic diseases. Applicant: Georg-August-Universität Göttingen Stiftung Öffentlichen Rechts, Universitätsmedizin Georg-August-Universität Göttingen Stiftung Öffentlichen Rechts. The sequence listing filed with the application follows.

SEQUENCE LISTING (6 sequences)

SEQ ID NO: 1 - DNA, 21 bp, Artificial Sequence
  artificial primer sequence (human GAPDH-F)
acccactcctccacctttgac

SEQ ID NO: 2 - DNA, 21 bp, Artificial Sequence
  artificial primer sequence (human GAPDH-R)
tccaccaccctgttgctgtag

SEQ ID NO: 3 - DNA, 24 bp, Artificial Sequence
  artificial primer sequence (human ACTA2-F)
actgagcgtggctattcctccgtt

SEQ ID NO: 4 - DNA, 21 bp, Artificial Sequence
  artificial primer sequence (human ACTA2-R)
gcagtggccatctcattttca

SEQ ID NO: 5 - DNA, 20 bp, Artificial Sequence
  artificial primer sequence (human Collagen 1-F)
gtactggattgaccccaacc

SEQ ID NO: 6 - DNA, 20 bp, Artificial Sequence
  artificial primer sequence (human Collagen 1-R)
cgccatactcgaactggaat